European Patent Specification EP 4 204 432 B1, published March 11, 2026. Title: METHODS AND COMPOSITIONS FOR PURIFICATION OF TRIMERIC FUSION PROTEINS. Applicant: Sichuan Clover Biopharmaceuticals, Inc. The sequence listing filed with the application follows.

SEQUENCE LISTING (46 sequences)

SEQ ID NO: 1 - protein, 1632 aa, Artificial Sequence
  Full length Endo180-Fc (D1-10-Fc)
MGPGRPAPAPWPRHLLRCVLLLGCLHLGRPGAPGDAALPEPNVFLIFSHGLQGCLEAQGGQVRVTPACNTSLPAQRWKWVSRNRLFNLGTMQCLGTGWPGTNTTASLGMYECDREALNLRWHCRTLGDQLSLLLGARTSNISKPGTLERGDQTRSGQWRIYGSEEDLCALPYHEVYTIQGNSHGKPCTIPFKYDNQWFHGCTSTGREDGHLWCATTQDYGKDERWGFCPIKSNDCETFWDKDQLTDSCYQFNFQSTLSWREAWASCEQQGADLLSITEIHEQTYINGLLTGYSSTLWIGLNDLDTSGGWQWSDNSPLKYLNWESDQPDNPSEENCGVIRTESSGGWQNRDCSIALPYVCKKKPNATAEPTPPDRWANVKVECEPSWQPFQGHCYRLQAEKRSWQESKKACLRGGGDLVSIHSMAELEFITKQIKQEVEELWIGLNDLKLQMNFEWSDGSLVSFTHWHPFEPNNFRDSLEDCVTIWGPEGRWNDSPCNQSLPSICKKAGQLSQGAAEEDHGCRKGWTWHSPSCYWLGEDQVTYSEARRLCTDHGSQLVTITNRFEQAFVSSLIYNWEGEYFWTALQDLNSTGSFFWLSGDEVMYTHWNRDQPGYSRGGCVALATGSAMGLWEVKNCTSFRARYICRQSLGTPVTPELPGPDPTPSLTGSCPQGWASDTKLRYCYKVFSSERLQDKKSWVQAQGACQELGAQLLSLASYEEEHFVANMLNKIFGESEPEIHEQHWFWIGLNRRDPRGGQSWRWSDGVGFSYHNFDRSRHDDDDIRGCAVLDLASLQWVAMQCDTQLDWICKIPRGTDVREPDDSPQGRREWLRFQEAEYKFFEHHSTWAQAQRICTWFQAELTSVHSQAELDFLSHNLQKFSRAQEQHWWIGLHTSESDGRFRWTDGSIINFISWAPGKPRPVGKDKKCVYMTASREDWGDQRCLTALPYICKRSNVTKETQPPDLPTTALGGCPSDWIQFLNKCFQVQGQEPQSRVKWSEAQFSCEQQEAQLVTITNPLEQAFITASLPNVTFDLWIGLHASQRDFQWVEQEPLMYANWAPGEPSGPSPAPSGNKPTSCAVVLHSPSAHFTGRWDDRSCTEETHGFICQKGTDPSLSPSPAALPPAPGTELSYLNGTFRLLQKPLRWHDALLLCESRNASLAYVPDPYTQAFLTQAARGLRTPLWIGLAGEEGSRRYSWVSEEPLNYVGWQDGEPQQPGGCTYVDVDGAWRTTSCDTKLQGAVCGVSSGPPPPRRISYHGSCPQGLADSAWIPFREHCYSFHMELLLGHKEARQRCQRAGGAVLSILDEMENVFVWEHLQSYEGQSRGAWLGMNFNPKGGTLVWQDNTAVNYSNWGPPGLGPSMLSHNSCYWIQSNSGLWRPGACTNITMGVVCKQAYVRSEPKSCDKTHTCPPCPAPELLGGPSVFLFPPKPKDTLMISRTPEVTCVVVDVSHEDPEVKFNWYVDGVEVHNAKTKPREEQYNSTYRVVSVLTVLHQDWLNGKEYKCKVSNKALPAPIEKTISKAKGQPREPQVYTLPPSRDELTKNQVSLTCLVKGFYPSDIAVEWESNGQPENNYKTTPPVLDSDGSFFLYSKLTVDKSRWQQGNVFSCSVMHEALHNHYTQKSLSLSPGK

SEQ ID NO: 2 - protein, 1602 aa, Artificial Sequence
  Mature Endo-180-Fc(D1-10-Fc)
GAPGDAALPEPNVFLIFSHGLQGCLEAQGGQVRVTPACNTSLPAQRWKWVSRNRLFNLGTMQCLGTGWPGTNTTASLGMYECDREALNLRWHCRTLGDQLSLLLGARTSNISKPGTLERGDQTRSGQWRIYGSEEDLCALPYHEVYTIQGNSHGKPCTIPFKYDNQWFHGCTSTGREDGHLWCATTQDYGKDERWGFCPIKSNDCETFWDKDQLTDSCYQFNFQSTLSWREAWASCEQQGADLLSITEIHEQTYINGLLTGYSSTLWIGLNDLDTSGGWQWSDNSPLKYLNWESDQPDNPSEENCGVIRTESSGGWQNRDCSIALPYVCKKKPNATAEPTPPDRWANVKVECEPSWQPFQGHCYRLQAEKRSWQESKKACLRGGGDLVSIHSMAELEFITKQIKQEVEELWIGLNDLKLQMNFEWSDGSLVSFTHWHPFEPNNFRDSLEDCVTIWGPEGRWNDSPCNQSLPSICKKAGQLSQGAAEEDHGCRKGWTWHSPSCYWLGEDQVTYSEARRLCTDHGSQLVTITNRFEQAFVSSLIYNWEGEYFWTALQDLNSTGSFFWLSGDEVMYTHWNRDQPGYSRGGCVALATGSAMGLWEVKNCTSFRARYICRQSLGTPVTPELPGPDPTPSLTGSCPQGWASDTKLRYCYKVFSSERLQDKKSWVQAQGACQELGAQLLSLASYEEEHFVANMLNKIFGESEPEIHEQHWFWIGLNRRDPRGGQSWRWSDGVGFSYHNFDRSRHDDDDIRGCAVLDLASLQWVAMQCDTQLDWICKIPRGTDVREPDDSPQGRREWLRFQEAEYKFFEHHSTWAQAQRICTWFQAELTSVHSQAELDFLSHNLQKFSRAQEQHWWIGLHTSESDGRFRWTDGSIINFISWAPGKPRPVGKDKKCVYMTASREDWGDQRCLTALPYICKRSNVTKETQPPDLPTTALGGCPSDWIQFLNKCFQVQGQEPQSRVKWSEAQFSCEQQEAQLVTITNPLEQAFITASLPNVTFDLWIGLHASQRDFQWVEQEPLMYANWAPGEPSGPSPAPSGNKPTSCAVVLHSPSAHFTGRWDDRSCTEETHGFICQKGTDPSLSPSPAALPPAPGTELSYLNGTFRLLQKPLRWHDALLLCESRNASLAYVPDPYTQAFLTQAARGLRTPLWIGLAGEEGSRRYSWVSEEPLNYVGWQDGEPQQPGGCTYVDVDGAWRTTSCDTKLQGAVCGVSSGPPPPRRISYHGSCPQGLADSAWIPFREHCYSFHMELLLGHKEARQRCQRAGGAVLSILDEMENVFVWEHLQSYEGQSRGAWLGMNFNPKGGTLVWQDNTAVNYSNWGPPGLGPSMLSHNSCYWIQSNSGLWRPGACTNITMGVVCKQAYVRSEPKSCDKTHTCPPCPAPELLGGPSVFLFPPKPKDTLMISRTPEVTCVVVDVSHEDPEVKFNWYVDGVEVHNAKTKPREEQYNSTYRVVSVLTVLHQDWLNGKEYKCKVSNKALPAPIEKTISKAKGQPREPQVYTLPPSRDELTKNQVSLTCLVKGFYPSDIAVEWESNGQPENNYKTTPPVLDSDGSFFLYSKLTVDKSRWQQGNVFSCSVMHEALHNHYTQKSLSLSPGK

SEQ ID NO: 3 - protein, 427 aa, Artificial Sequence
  Full Length D6-Fc
MGPGRPAPAPWPRHLLRCVLLLGCLHLGRPRSPVTPELPGPDPTPSLTGSCPQGWASDTKLRYCYKVFSSERLQDKKSWVQAQGACQELGAQLLSLASYEEEHFVANMLNKIFGESEPEIHEQHWFWIGLNRRDPRGGQSWRWSDGVGFSYHNFDRSRHDDDDIRGCAVLDLASLQWVAMQCDTQLDWICKIPRSEPKSCDKTHTCPPCPAPELLGGPSVFLFPPKPKDTLMISRTPEVTCVVVDVSHEDPEVKFNWYVDGVEVHNAKTKPREEQYNSTYRVVSVLTVLHQDWLNGKEYKCKVSNKALPAPIEKTISKAKGQPREPQVYTLPPSRDELTKNQVSLTCLVKGFYPSDIAVEWESNGQPENNYKTTPPVLDSDGSFFLYSKLTVDKSRWQQGNVFSCSVMHEALHNHYTQKSLSLSPGK

SEQ ID NO: 4 - protein, 397 aa, Artificial Sequence
  Mature D6-Fc
RSPVTPELPGPDPTPSLTGSCPQGWASDTKLRYCYKVFSSERLQDKKSWVQAQGACQELGAQLLSLASYEEEHFVANMLNKIFGESEPEIHEQHWFWIGLNRRDPRGGQSWRWSDGVGFSYHNFDRSRHDDDDIRGCAVLDLASLQWVAMQCDTQLDWICKIPRSEPKSCDKTHTCPPCPAPELLGGPSVFLFPPKPKDTLMISRTPEVTCVVVDVSHEDPEVKFNWYVDGVEVHNAKTKPREEQYNSTYRVVSVLTVLHQDWLNGKEYKCKVSNKALPAPIEKTISKAKGQPREPQVYTLPPSRDELTKNQVSLTCLVKGFYPSDIAVEWESNGQPENNYKTTPPVLDSDGSFFLYSKLTVDKSRWQQGNVFSCSVMHEALHNHYTQKSLSLSPGK

SEQ ID NO: 5 - protein, 30 aa, Artificial Sequence
  Signal Peptide
MGPGRPAPAPWPRHLLRCVLLLGCLHLGRP

SEQ ID NO: 6 - protein, 232 aa, Artificial Sequence
  Fc
EPKSCDKTHTCPPCPAPELLGGPSVFLFPPKPKDTLMISRTPEVTCVVVDVSHEDPEVKFNWYVDGVEVHNAKTKPREEQYNSTYRVVSVLTVLHQDWLNGKEYKCKVSNKALPAPIEKTISKAKGQPREPQVYTLPPSRDELTKNQVSLTCLVKGFYPSDIAVEWESNGQPENNYKTTPPVLDSDGSFFLYSKLTVDKSRWQQGNVFSCSVMHEALHNHYTQKSLSLSPGK

SEQ ID NO: 7 - protein, 1384 aa, Artificial Sequence
  Mature Endo180 Ecto-domain (Uniprot Q9UBG0)
GAPGDAALPEPNVFLIFSHGLQGCLEAQGGQVRVTPACNTSLPAQRWKWVSRNRLFNLGTMQCLGTGWPGTNTTASLGMYECDREALNLRWHCRTLGDQLSLLLGARTSNISKPGTLERGDQTRSGQWRIYGSEEDLCALPYHEVYTIQGNSHGKPCTIPFKYDNQWFHGCTSTGREDGHLWCATTQDYGKDERWGFCPIKSNDCETFWDKDQLTDSCYQFNFQSTLSWREAWASCEQQGADLLSITEIHEQTYINGLLTGYSSTLWIGLNDLDTSGGWQWSDNSPLKYLNWESDQPDNPSEENCGVIRTESSGGWQNRDCSIALPYVCKKKPNATAEPTPPDRWANVKVECEPSWQPFQGHCYRLQAEKRSWQESKKACLRGGGDLVSIHSMAELEFITKQIKQEVEELWIGLNDLKLQMNFEWSDGSLVSFTHWHPFEPNNFRDSLEDCVTIWGPEGRWNDSPCNQSLPSICKKAGQLSQGAAEEDHGCRKGWTWHSPSCYWLGEDQVTYSEARRLCTDHGSQLVTITNRFEQAFVSSLIYNWEGEYFWTALQDLNSTGSFFWLSGDEVMYTHWNRDQPGYSRGGCVALATGSAMGLWEVKNCTSFRARYICRQSLGTPVTPELPGPDPTPSLTGSCPQGWASDTKLRYCYKVFSSERLQDKKSWVQAQGACQELGAQLLSLASYEEEHFVANMLNKIFGESEPEIHEQHWFWIGLNRRDPRGGQSWRWSDGVGFSYHNFDRSRHDDDDIRGCAVLDLASLQWVAMQCDTQLDWICKIPRGTDVREPDDSPQGRREWLRFQEAEYKFFEHHSTWAQAQRICTWFQAELTSVHSQAELDFLSHNLQKFSRAQEQHWWIGLHTSESDGRFRWTDGSIINFISWAPGKPRPVGKDKKCVYMTASREDWGDQRCLTALPYICKRSNVTKETQPPDLPTTALGGCPSDWIQFLNKCFQVQGQEPQSRVKWSEAQFSCEQQEAQLVTITNPLEQAFITASLPNVTFDLWIGLHASQRDFQWVEQEPLMYANWAPGEPSGPSPAPSGNKPTSCAVVLHSPSAHFTGRWDDRSCTEETHGFICQKGTDPSLSPSPAALPPAPGTELSYLNGTFRLLQKPLRWHDALLLCESRNASLAYVPDPYTQAFLTQAARGLRTPLWIGLAGEEGSRRYSWVSEEPLNYVGWQDGEPQQPGGCTYVDVDGAWRTTSCDTKLQGAVCGVSSGPPPPRRISYHGSCPQGLADSAWIPFREHCYSFHMELLLGHKEARQRCQRAGGAVLSILDEMENVFVWEHLQSYEGQSRGAWLGMNFNPKGGTLVWQDNTAVNYSNWGPPGLGPSMLSHNSCYWIQSNSGLWRPGACTNITMGVVCKLPRAEQSSFSPSALPENPAA

SEQ ID NO: 8 - protein, 127 aa, Artificial Sequence
  D1 (Ricin B-type lectin domain)
PNVFLIFSHGLQGCLEAQGGQVRVTPACNTSLPAQRWKWVSRNRLFNLGTMQCLGTGWPGTNTTASLGMYECDREALNLRWHCRTLGDQLSLLLGARTSNISKPGTLERGDQTRSGQWRIYGSEEDL

SEQ ID NO: 9 - protein, 49 aa, Artificial Sequence
  D2 (Fibronectin type-II domain)
SHGKPCTIPFKYDNQWFHGCTSTGREDGHLWCATTQDYGKDERWGFCPI

SEQ ID NO: 10 - protein, 117 aa, Artificial Sequence
  D3 (C-type lectin 1)
LTDSCYQFNFQSTLSWREAWASCEQQGADLLSITEIHEQTYINGLLTGYSSTLWIGLNDLDTSGGWQWSDNSPLKYLNWESDQPDNPSEENCGVIRTESSGGWQNRDCSIALPYVCK

SEQ ID NO: 11 - protein, 117 aa, Artificial Sequence
  D4 (C-type lectin 2)
FQGHCYRLQAEKRSWQESKKACLRGGGDLVSIHSMAELEFITKQIKQEVEELWIGLNDLKLQMNFEWSDGSLVSFTHWHPFEPNNFRDSLEDCVTIWGPEGRWNDSPCNQSLPSICK

SEQ ID NO: 12 - protein, 117 aa, Artificial Sequence
  D5 (C-type lectin 3)
HSPSCYWLGEDQVTYSEARRLCTDHGSQLVTITNRFEQAFVSSLIYNWEGEYFWTALQDLNSTGSFFWLSGDEVMYTHWNRDQPGYSRGGCVALATGSAMGLWEVKNCTSFRARYIC

SEQ ID NO: 13 - protein, 132 aa, Artificial Sequence
  D6 (C-type lectin 4)
KLRYCYKVFSSERLQDKKSWVQAQGACQELGAQLLSLASYEEEHFVANMLNKIFGESEPEIHEQHWFWIGLNRRDPRGGQSWRWSDGVGFSYHNFDRSRHDDDDIRGCAVLDLASLQWVAMQCDTQLDWICK

SEQ ID NO: 14 - protein, 120 aa, Artificial Sequence
  D7 (C-type lectin 5)
FQEAEYKFFEHHSTWAQAQRICTWFQAELTSVHSQAELDFLSHNLQKFSRAQEQHWWIGLHTSESDGRFRWTDGSIINFISWAPGKPRPVGKDKKCVYMTASREDWGDQRCLTALPYICK

SEQ ID NO: 15 - protein, 129 aa, Artificial Sequence
  D8 (C-type lectin 6)
FLNKCFQVQGQEPQSRVKWSEAQFSCEQQEAQLVTITNPLEQAFITASLPNVTFDLWIGLHASQRDFQWVEQEPLMYANWAPGEPSGPSPAPSGNKPTSCAVVLHSPSAHFTGRWDDRSCTEETHGFIC

SEQ ID NO: 16 - protein, 112 aa, Artificial Sequence
  D9 (C-type lectin 7)
YLNGTFRLLQKPLRWHDALLLCESRNASLAYVPDPYTQAFLTQAARGLRTPLWIGLAGEEGSRRYSWVSEEPLNYVGWQDGEPQQPGGCTYVDVDGAWRTTSCDTKLQGAVC

SEQ ID NO: 17 - protein, 121 aa, Artificial Sequence
  D10 (C-type lectin 8)
FREHCYSFHMELLLGHKEARQRCQRAGGAVLSILDEMENVFVWEHLQSYEGQSRGAWLGMNFNPKGGTLVWQDNTAVNYSNWGPPGLGPSMLSHNSCYWIQSNSGLWRPGACTNITMGVVC

SEQ ID NO: 18 - protein, 309 aa, Artificial Sequence
  Trimerization peptide (Type I) with glycine-X-Y repeats and D→N mutation at BMP-1 site, KS version
NGLPGPIGPPGPRGRTGDAGPVGPPGPPGPPGPPGPPSAGFDFSFLPQPPQEKAHDGGRYYRANDANVVRDRDLEVDTTLKSLSQQIENIRSPEGSRKNPARTCRDLKMCHSDWKSGEYWIDPNQGCNLDAIKVFCNMETGETCVYPTQPSVAQKNWYISKNPKDKRHVWFGESMTDGFQFEYGGQGSDPADVAIQLTFLRLMSTEASQNITYHCKNSVAYMDQQTGNLKKALLLKGSNEIEIRAEGNSRFTYSVTVDGCTSHTGAWGKTVIEYKTTKSSRLPIIDVAPLDVGAPDQEFGFDVGPVCFL

SEQ ID NO: 19 - protein, 309 aa, Artificial Sequence
  Trimerization peptide (Type I) with glycine-X-Y repeats and A→N mutation at BMP-1 site, KS version
NGLPGPIGPPGPRGRTGDAGPVGPPGPPGPPGPPGPPSAGFDFSFLPQPPQEKAHDGGRYYRNDDANVVRDRDLEVDTTLKSLSQQIENIRSPEGSRKNPARTCRDLKMCHSDWKSGEYWIDPNQGCNLDAIKVFCNMETGETCVYPTQPSVAQKNWYISKNPKDKRHVWFGESMTDGFQFEYGGQGSDPADVAIQLTFLRLMSTEASQNITYHCKNSVAYMDQQTGNLKKALLLKGSNEIEIRAEGNSRFTYSVTVDGCTSHTGAWGKTVIEYKTTKSSRLPIIDVAPLDVGAPDQEFGFDVGPVCFL

SEQ ID NO: 20 - protein, 311 aa, Artificial Sequence
  Trimerization peptide (Type I) with glycine-X-Y repeats and D→N mutation at BMP-1 site, KS version
RSNGLPGPIGPPGPRGRTGDAGPVGPPGPPGPPGPPGPPSAGFDFSFLPQPPQEKAHDGGRYYRANDANVVRDRDLEVDTTLKSLSQQIENIRSPEGSRKNPARTCRDLKMCHSDWKSGEYWIDPNQGCNLDAIKVFCNMETGETCVYPTQPSVAQKNWYISKNPKDKRHVWFGESMTDGFQFEYGGQGSDPADVAIQLTFLRLMSTEASQNITYHCKNSVAYMDQQTGNLKKALLLKGSNEIEIRAEGNSRFTYSVTVDGCTSHTGAWGKTVIEYKTTKSSRLPIIDVAPLDVGAPDQEFGFDVGPVCFL

SEQ ID NO: 21 - protein, 311 aa, Artificial Sequence
  Trimerization peptide (Type I) with glycine-X-Y repeats and D→N mutation at BMP-1 site, KS version
GSNGLPGPIGPPGPRGRTGDAGPVGPPGPPGPPGPPGPPSAGFDFSFLPQPPQEKAHDGGRYYRANDANVVRDRDLEVDTTLKSLSQQIENIRSPEGSRKNPARTCRDLKMCHSDWKSGEYWIDPNQGCNLDAIKVFCNMETGETCVYPTQPSVAQKNWYISKNPKDKRHVWFGESMTDGFQFEYGGQGSDPADVAIQLTFLRLMSTEASQNITYHCKNSVAYMDQQTGNLKKALLLKGSNEIEIRAEGNSRFTYSVTVDGCTSHTGAWGKTVIEYKTTKSSRLPIIDVAPLDVGAPDQEFGFDVGPVCFL

SEQ ID NO: 22 - protein, 309 aa, Artificial Sequence
  Trimerization peptide (Type I) with glycine-X-Y repeats, no BMP-1 site mutation, KS version
NGLPGPIGPPGPRGRTGDAGPVGPPGPPGPPGPPGPPSAGFDFSFLPQPPQEKAHDGGRYYRADDANVVRDRDLEVDTTLKSLSQQIENIRSPEGSRKNPARTCRDLKMCHSDWKSGEYWIDPNQGCNLDAIKVFCNMETGETCVYPTQPSVAQKNWYISKNPKDKRHVWFGESMTDGFQFEYGGQGSDPADVAIQLTFLRLMSTEASQNITYHCKNSVAYMDQQTGNLKKALLLKGSNEIEIRAEGNSRFTYSVTVDGCTSHTGAWGKTVIEYKTTKSSRLPIIDVAPLDVGAPDQEFGFDVGPVCFL

SEQ ID NO: 23 - protein, 310 aa, Artificial Sequence
  Trimerization peptide (Type I) with glycine-X-Y repeats, no BMP-1 site mutation, KS version
SNGLPGPIGPPGPRGRTGDAGPVGPPGPPGPPGPPGPPSAGFDFSFLPQPPQEKAHDGGRYYRADDANVVRDRDLEVDTTLKSLSQQIENIRSPEGSRKNPARTCRDLKMCHSDWKSGEYWIDPNQGCNLDAIKVFCNMETGETCVYPTQPSVAQKNWYISKNPKDKRHVWFGESMTDGFQFEYGGQGSDPADVAIQLTFLRLMSTEASQNITYHCKNSVAYMDQQTGNLKKALLLKGSNEIEIRAEGNSRFTYSVTVDGCTSHTGAWGKTVIEYKTTKSSRLPIIDVAPLDVGAPDQEFGFDVGPVCFL

SEQ ID NO: 24 - protein, 309 aa, Artificial Sequence
  Trimerization peptide (Type I) with glycine-X-Y repeats, no BMP-1 site mutation, QT version
NGLPGPIGPPGPRGRTGDAGPVGPPGPPGPPGPPGPPSAGFDFSFLPQPPQEKAHDGGRYYRADDANVVRDRDLEVDTTLKSLSQQIENIRSPEGSRKNPARTCRDLKMCHSDWKSGEYWIDPNQGCNLDAIKVFCNMETGETCVYPTQPSVAQKNWYISKNPKDKRHVWFGESMTDGFQFEYGGQGSDPADVAIQLTFLRLMSTEASQNITYHCKNSVAYMDQQTGNLKKALLLQGSNEIEIRAEGNSRFTYSVTVDGCTSHTGAWGKTVIEYKTTKTSRLPIIDVAPLDVGAPDQEFGFDVGPVCFL

SEQ ID NO: 25 - protein, 310 aa, Artificial Sequence
  Trimerization peptide (Type I) with glycine-X-Y repeats, no BMP-1 site mutation, QT version
SNGLPGPIGPPGPRGRTGDAGPVGPPGPPGPPGPPGPPSAGFDFSFLPQPPQEKAHDGGRYYRADDANVVRDRDLEVDTTLKSLSQQIENIRSPEGSRKNPARTCRDLKMCHSDWKSGEYWIDPNQGCNLDAIKVFCNMETGETCVYPTQPSVAQKNWYISKNPKDKRHVWFGESMTDGFQFEYGGQGSDPADVAIQLTFLRLMSTEASQNITYHCKNSVAYMDQQTGNLKKALLLQGSNEIEIRAEGNSRFTYSVTVDGCTSHTGAWGKTVIEYKTTKTSRLPIIDVAPLDVGAPDQEFGFDVGPVCFL

SEQ ID NO: 26 - protein, 244 aa, Artificial Sequence
  Trimerization peptide (Type I), KS version
ANVVRDRDLEVDTTLKSLSQQIENIRSPEGSRKNPARTCRDLKMCHSDWKSGEYWIDPNQGCNLDAIKVFCNMETGETCVYPTQPSVAQKNWYISKNPKDKRHVWFGESMTDGFQFEYGGQGSDPADVAIQLTFLRLMSTEASQNITYHCKNSVAYMDQQTGNLKKALLLKGSNEIEIRAEGNSRFTYSVTVDGCTSHTGAWGKTVIEYKTTKSSRLPIIDVAPLDVGAPDQEFGFDVGPVCFL

SEQ ID NO: 27 - protein, 244 aa, Artificial Sequence
  Trimerization peptide (Type I), KS version
DANVVRDRDLEVDTTLKSLSQQIENIRSPEGSRKNPARTCRDLKMCHSDWKSGEYWIDPNQGCNLDAIKVFCNMETGETCVYPTQPSVAQKNWYISKNPKDKRHVWFGESMTDGFQFEYGGQGSDPADVAIQLTFLRLMSTEASQNITYHCKNSVAYMDQQTGNLKKALLLKGSNEIEIRAEGNSRFTYSVTVDGCTSHTGAWGKTVIEYKTTKSSRLPIIDVAPLDVGAPDQEFGFDVGPVCF

SEQ ID NO: 28 - protein, 246 aa, Artificial Sequence
  Trimerization peptide (Type I), KS version
SDANVVRDRDLEVDTTLKSLSQQIENIRSPEGSRKNPARTCRDLKMCHSDWKSGEYWIDPNQGCNLDAIKVFCNMETGETCVYPTQPSVAQKNWYISKNPKDKRHVWFGESMTDGFQFEYGGQGSDPADVAIQLTFLRLMSTEASQNITYHCKNSVAYMDQQTGNLKKALLLKGSNEIEIRAEGNSRFTYSVTVDGCTSHTGAWGKTVIEYKTTKSSRLPIIDVAPLDVGAPDQEFGFDVGPVCFL

SEQ ID NO: 29 - protein, 247 aa, Artificial Sequence
  Trimerization peptide (Type I), KS version
RSDANVVRDRDLEVDTTLKSLSQQIENIRSPEGSRKNPARTCRDLKMCHSDWKSGEYWIDPNQGCNLDAIKVFCNMETGETCVYPTQPSVAQKNWYISKNPKDKRHVWFGESMTDGFQFEYGGQGSDPADVAIQLTFLRLMSTEASQNITYHCKNSVAYMDQQTGNLKKALLLKGSNEIEIRAEGNSRFTYSVTVDGCTSHTGAWGKTVIEYKTTKSSRLPIIDVAPLDVGAPDQEFGFDVGPVCFL

SEQ ID NO: 30 - protein, 309 aa, Artificial Sequence
  Trimerization peptide (Type I), with glycine-X-Y repeats and D→N mutation at BMP-1 site, QT version
NGLPGPIGPPGPRGRTGDAGPVGPPGPPGPPGPPGPPSAGFDFSFLPQPPQEKAHDGGRYYRANDANVVRDRDLEVDTTLKSLSQQIENIRSPEGSRKNPARTCRDLKMCHSDWKSGEYWIDPNQGCNLDAIKVFCNMETGETCVYPTQPSVAQKNWYISKNPKDKRHVWFGESMTDGFQFEYGGQGSDPADVAIQLTFLRLMSTEASQNITYHCKNSVAYMDQQTGNLKKALLLQGSNEIEIRAEGNSRFTYSVTVDGCTSHTGAWGKTVIEYKTTKTSRLPIIDVAPLDVGAPDQEFGFDVGPVCFL

SEQ ID NO: 31 - protein, 309 aa, Artificial Sequence
  Trimerization peptide (Type I), with glycine-X-Y repeats and A→N mutation at BMP-1 site, QT version
NGLPGPIGPPGPRGRTGDAGPVGPPGPPGPPGPPGPPSAGFDFSFLPQPPQEKAHDGGRYYRNDDANVVRDRDLEVDTTLKSLSQQIENIRSPEGSRKNPARTCRDLKMCHSDWKSGEYWIDPNQGCNLDAIKVFCNMETGETCVYPTQPSVAQKNWYISKNPKDKRHVWFGESMTDGFQFEYGGQGSDPADVAIQLTFLRLMSTEASQNITYHCKNSVAYMDQQTGNLKKALLLQGSNEIEIRAEGNSRFTYSVTVDGCTSHTGAWGKTVIEYKTTKTSRLPIIDVAPLDVGAPDQEFGFDVGPVCFL

SEQ ID NO: 32 - protein, 311 aa, Artificial Sequence
  Trimerization peptide (Type I), with glycine-X-Y repeats and D→N mutation at BMP-1 site, QT version
RSNGLPGPIGPPGPRGRTGDAGPVGPPGPPGPPGPPGPPSAGFDFSFLPQPPQEKAHDGGRYYRANDANVVRDRDLEVDTTLKSLSQQIENIRSPEGSRKNPARTCRDLKMCHSDWKSGEYWIDPNQGCNLDAIKVFCNMETGETCVYPTQPSVAQKNWYISKNPKDKRHVWFGESMTDGFQFEYGGQGSDPADVAIQLTFLRLMSTEASQNITYHCKNSVAYMDQQTGNLKKALLLQGSNEIEIRAEGNSRFTYSVTVDGCTSHTGAWGKTVIEYKTTKTSRLPIIDVAPLDVGAPDQEFGFDVGPVCFL

SEQ ID NO: 33 - protein, 311 aa, Artificial Sequence
  Trimerization peptide (Type I), with glycine-X-Y repeats and D→N mutation at BMP-1 site, QT version
GSNGLPGPIGPPGPRGRTGDAGPVGPPGPPGPPGPPGPPSAGFDFSFLPQPPQEKAHDGGRYYRANDANVVRDRDLEVDTTLKSLSQQIENIRSPEGSRKNPARTCRDLKMCHSDWKSGEYWIDPNQGCNLDAIKVFCNMETGETCVYPTQPSVAQKNWYISKNPKDKRHVWFGESMTDGFQFEYGGQGSDPADVAIQLTFLRLMSTEASQNITYHCKNSVAYMDQQTGNLKKALLLQGSNEIEIRAEGNSRFTYSVTVDGCTSHTGAWGKTVIEYKTTKTSRLPIIDVAPLDVGAPDQEFGFDVGPVCFL

SEQ ID NO: 34 - protein, 234 aa, Artificial Sequence
  Trimerization peptide (Type III)
DEIMTSLKSVNGQIESLISPDGSRKNPARNCRDLKFCHPELKSGEYWVDPNQGCKLDAIKVFCNMETGETCISANPLNVPRKHWWTDSSAEKKHVWFGESMDGGFQFSYGNPELPEDVLDVQLAFLRLLSSRASQNITYHCKNSIAYMDQASGNVKKALKLMGSNEGEFKAEGNSKFTYTVLEDGCTKHTGEWSKTVFEYRTRKAVRLPIVDIAPYDIGGPDQEFGVDVGPVCF

SEQ ID NO: 35 - protein, 244 aa, Artificial Sequence
  Trimerization peptide (Type III)
EPMDFKINTDEIMTSLKSVNGQIESLISPDGSRKNPARNCRDLKFCHPELKSGEYWVDPNQGCKLDAIKVFCNMETGETCISANPLNVPRKHWWTDSSAEKKHVWFGESMDGGFQFSYGNPELPEDVLDVQLAFLRLLSSRASQNITYHCKNSIAYMDQASGNVKKALKLMGSNEGEFKAEGNSKFTYTVLEDGCTKHTGEWSKTVFEYRTRKAVRLPIVDIAPYDIGGPDQEFGVDVGPVCFL

SEQ ID NO: 36 - protein, 245 aa, Artificial Sequence
  Trimerization peptide (Type III)
SEPMDFKINTDEIMTSLKSVNGQIESLISPDGSRKNPARNCRDLKFCHPELKSGEYWVDPNQGCKLDAIKVFCNMETGETCISANPLNVPRKHWWTDSSAEKKHVWFGESMDGGFQFSYGNPELPEDVLDVQLAFLRLLSSRASQNITYHCKNSIAYMDQASGNVKKALKLMGSNEGEFKAEGNSKFTYTVLEDGCTKHTGEWSKTVFEYRTRKAVRLPIVDIAPYDIGGPDQEFGVDVGPVCFL

SEQ ID NO: 37 - protein, 246 aa, Artificial Sequence
  Trimerization peptide (Type III)
RSEPMDFKINTDEIMTSLKSVNGQIESLISPDGSRKNPARNCRDLKFCHPELKSGEYWVDPNQGCKLDAIKVFCNMETGETCISANPLNVPRKHWWTDSSAEKKHVWFGESMDGGFQFSYGNPELPEDVLDVQLAFLRLLSSRASQNITYHCKNSIAYMDQASGNVKKALKLMGSNEGEFKAEGNSKFTYTVLEDGCTKHTGEWSKTVFEYRTRKAVRLPIVDIAPYDIGGPDQEFGVDVGPVCFL

SEQ ID NO: 38 - protein, 244 aa, Artificial Sequence
  Trimerization peptide (Type I), QT version
ANVVRDRDLEVDTTLKSLSQQIENIRSPEGSRKNPARTCRDLKMCHSDWKSGEYWIDPNQGCNLDAIKVFCNMETGETCVYPTQPSVAQKNWYISKNPKDKRHVWFGESMTDGFQFEYGGQGSDPADVAIQLTFLRLMSTEASQNITYHCKNSVAYMDQQTGNLKKALLLQGSNEIEIRAEGNSRFTYSVTVDGCTSHTGAWGKTVIEYKTTKTSRLPIIDVAPLDVGAPDQEFGFDVGPVCFL

SEQ ID NO: 39 - protein, 246 aa, Artificial Sequence
  Trimerization peptide (Type I), QT version
SDANVVRDRDLEVDTTLKSLSQQIENIRSPEGSRKNPARTCRDLKMCHSDWKSGEYWIDPNQGCNLDAIKVFCNMETGETCVYPTQPSVAQKNWYISKNPKDKRHVWFGESMTDGFQFEYGGQGSDPADVAIQLTFLRLMSTEASQNITYHCKNSVAYMDQQTGNLKKALLLQGSNEIEIRAEGNSRFTYSVTVDGCTSHTGAWGKTVIEYKTTKTSRLPIIDVAPLDVGAPDQEFGFDVGPVCFL

SEQ ID NO: 40 - protein, 247 aa, Artificial Sequence
  Trimerization peptide (Type I), QT version
RSDANVVRDRDLEVDTTLKSLSQQIENIRSPEGSRKNPARTCRDLKMCHSDWKSGEYWIDPNQGCNLDAIKVFCNMETGETCVYPTQPSVAQKNWYISKNPKDKRHVWFGESMTDGFQFEYGGQGSDPADVAIQLTFLRLMSTEASQNITYHCKNSVAYMDQQTGNLKKALLLQGSNEIEIRAEGNSRFTYSVTVDGCTSHTGAWGKTVIEYKTTKTSRLPIIDVAPLDVGAPDQEFGFDVGPVCFL

SEQ ID NO: 41 - protein, 247 aa, Artificial Sequence
  Trimerization peptide (Type I), QT version
GSDANVVRDRDLEVDTTLKSLSQQIENIRSPEGSRKNPARTCRDLKMCHSDWKSGEYWIDPNQGCNLDAIKVFCNMETGETCVYPTQPSVAQKNWYISKNPKDKRHVWFGESMTDGFQFEYGGQGSDPADVAIQLTFLRLMSTEASQNITYHCKNSVAYMDQQTGNLKKALLLQGSNEIEIRAEGNSRFTYSVTVDGCTSHTGAWGKTVIEYKTTKTSRLPIIDVAPLDVGAPDQEFGFDVGPVCFL

SEQ ID NO: 42 - protein, 234 aa, Artificial Sequence
  Fc
RVEPKSCDKTHTCPPCPAPELLGGPSVFLFPPKPKDTLMISRTPEVTCVVVDVSHEDPEVKFNWYVDGVEVHNAKTKPREEQYNSTYRVVSVLTVLHQDWLNGKEYKCKVSNKALPAPIEKTISKAKGQPREPQVYTLPPSRDELTKNQVSLTCLVKGFYPSDIAVEWESNGQPENNYKTTPPVLDSDGSFFLYSKLTVDKSRWQQGNVFSCSVMHEALHNHYTQKSLSLSPGK

SEQ ID NO: 43 - protein, 1628 aa, Artificial Sequence
  Full length Endo180-Fc (D1-10-Fc)
MGPGRPAPAPWPRHLLRCVLLLGCLHLGRPGAPGDAALPEPNVFLIFSHGLQGCLEAQGGQVRVTPACNTSLPAQRWKWVSRNRLFNLGTMQCLGTGWPGTNTTASLGMYECDREALNLRWHCRTLGDQLSLLLGARTSNISKPGTLERGDQTRSGQWRIYGSEEDLCALPYHEVYTIQGNSHGKPCTIPFKYDNQWFHGCTSTGREDGHLWCATTQDYGKDERWGFCPIKSNDCETFWDKDQLTDSCYQFNFQSTLSWREAWASCEQQGADLLSITEIHEQTYINGLLTGYSSTLWIGLNDLDTSGGWQWSDNSPLKYLNWESDQPDNPSEENCGVIRTESSGGWQNRDCSIALPYVCKKKPNATAEPTPPDRWANVKVECEPSWQPFQGHCYRLQAEKRSWQESKKACLRGGGDLVSIHSMAELEFITKQIKQEVEELWIGLNDLKLQMNFEWSDGSLVSFTHWHPFEPNNFRDSLEDCVTIWGPEGRWNDSPCNQSLPSICKKAGQLSQGAAEEDHGCRKGWTWHSPSCYWLGEDQVTYSEARRLCTDHGSQLVTITNRFEQAFVSSLIYNWEGEYFWTALQDLNSTGSFFWLSGDEVMYTHWNRDQPGYSRGGCVALATGSAMGLWEVKNCTSFRARYICRQSLGTPVTPELPGPDPTPSLTGSCPQGWASDTKLRYCYKVFSSERLQDKKSWVQAQGACQELGAQLLSLASYEEEHFVANMLNKIFGESEPEIHEQHWFWIGLNRRDPRGGQSWRWSDGVGFSYHNFDRSRHDDDDIRGCAVLDLASLQWVAMQCDTQLDWICKIPRGTDVREPDDSPQGRREWLRFQEAEYKFFEHHSTWAQAQRICTWFQAELTSVHSQAELDFLSHNLQKFSRAQEQHWWIGLHTSESDGRFRWTDGSIINFISWAPGKPRPVGKDKKCVYMTASREDWGDQRCLTALPYICKRSNVTKETQPPDLPTTALGGCPSDWIQFLNKCFQVQGQEPQSRVKWSEAQFSCEQQEAQLVTITNPLEQAFITASLPNVTFDLWIGLHASQRDFQWVEQEPLMYANWAPGEPSGPSPAPSGNKPTSCAVVLHSPSAHFTGRWDDRSCTEETHGFICQKGTDPSLSPSPAALPPAPGTELSYLNGTFRLLQKPLRWHDALLLCESRNASLAYVPDPYTQAFLTQAARGLRTPLWIGLAGEEGSRRYSWVSEEPLNYVGWQDGEPQQPGGCTYVDVDGAWRTTSCDTKLQGAVCGVSSGPPPPRRISYHGSCPQGLADSAWIPFREHCYSFHMELLLGHKEARQRCQRAGGAVLSILDEMENVFVWEHLQSYEGQSRGAWLGMNFNPKGGTLVWQDNTAVNYSNWGPPGLGPSMLSHNSCYWIQSNSGLWRPGACTNITMGVVCKRVEPKSCDKTHTCPPCPAPELLGGPSVFLFPPKPKDTLMISRTPEVTCVVVDVSHEDPEVKFNWYVDGVEVHNAKTKPREEQYNSTYRVVSVLTVLHQDWLNGKEYKCKVSNKALPAPIEKTISKAKGQPREPQVYTLPPSRDELTKNQVSLTCLVKGFYPSDIAVEWESNGQPENNYKTTPPVLDSDGSFFLYSKLTVDKSRWQQGNVFSCSVMHEALHNHYTQKSLSLSPGK

SEQ ID NO: 44 - protein, 1598 aa, Artificial Sequence
  Mature Endo-180-Fc(D1-10-Fc)
GAPGDAALPEPNVFLIFSHGLQGCLEAQGGQVRVTPACNTSLPAQRWKWVSRNRLFNLGTMQCLGTGWPGTNTTASLGMYECDREALNLRWHCRTLGDQLSLLLGARTSNISKPGTLERGDQTRSGQWRIYGSEEDLCALPYHEVYTIQGNSHGKPCTIPFKYDNQWFHGCTSTGREDGHLWCATTQDYGKDERWGFCPIKSNDCETFWDKDQLTDSCYQFNFQSTLSWREAWASCEQQGADLLSITEIHEQTYINGLLTGYSSTLWIGLNDLDTSGGWQWSDNSPLKYLNWESDQPDNPSEENCGVIRTESSGGWQNRDCSIALPYVCKKKPNATAEPTPPDRWANVKVECEPSWQPFQGHCYRLQAEKRSWQESKKACLRGGGDLVSIHSMAELEFITKQIKQEVEELWIGLNDLKLQMNFEWSDGSLVSFTHWHPFEPNNFRDSLEDCVTIWGPEGRWNDSPCNQSLPSICKKAGQLSQGAAEEDHGCRKGWTWHSPSCYWLGEDQVTYSEARRLCTDHGSQLVTITNRFEQAFVSSLIYNWEGEYFWTALQDLNSTGSFFWLSGDEVMYTHWNRDQPGYSRGGCVALATGSAMGLWEVKNCTSFRARYICRQSLGTPVTPELPGPDPTPSLTGSCPQGWASDTKLRYCYKVFSSERLQDKKSWVQAQGACQELGAQLLSLASYEEEHFVANMLNKIFGESEPEIHEQHWFWIGLNRRDPRGGQSWRWSDGVGFSYHNFDRSRHDDDDIRGCAVLDLASLQWVAMQCDTQLDWICKIPRGTDVREPDDSPQGRREWLRFQEAEYKFFEHHSTWAQAQRICTWFQAELTSVHSQAELDFLSHNLQKFSRAQEQHWWIGLHTSESDGRFRWTDGSIINFISWAPGKPRPVGKDKKCVYMTASREDWGDQRCLTALPYICKRSNVTKETQPPDLPTTALGGCPSDWIQFLNKCFQVQGQEPQSRVKWSEAQFSCEQQEAQLVTITNPLEQAFITASLPNVTFDLWIGLHASQRDFQWVEQEPLMYANWAPGEPSGPSPAPSGNKPTSCAVVLHSPSAHFTGRWDDRSCTEETHGFICQKGTDPSLSPSPAALPPAPGTELSYLNGTFRLLQKPLRWHDALLLCESRNASLAYVPDPYTQAFLTQAARGLRTPLWIGLAGEEGSRRYSWVSEEPLNYVGWQDGEPQQPGGCTYVDVDGAWRTTSCDTKLQGAVCGVSSGPPPPRRISYHGSCPQGLADSAWIPFREHCYSFHMELLLGHKEARQRCQRAGGAVLSILDEMENVFVWEHLQSYEGQSRGAWLGMNFNPKGGTLVWQDNTAVNYSNWGPPGLGPSMLSHNSCYWIQSNSGLWRPGACTNITMGVVCKRVEPKSCDKTHTCPPCPAPELLGGPSVFLFPPKPKDTLMISRTPEVTCVVVDVSHEDPEVKFNWYVDGVEVHNAKTKPREEQYNSTYRVVSVLTVLHQDWLNGKEYKCKVSNKALPAPIEKTISKAKGQPREPQVYTLPPSRDELTKNQVSLTCLVKGFYPSDIAVEWESNGQPENNYKTTPPVLDSDGSFFLYSKLTVDKSRWQQGNVFSCSVMHEALHNHYTQKSLSLSPGK

SEQ ID NO: 45 - protein, 427 aa, Artificial Sequence
  Full Length D6-Fc
MGPGRPAPAPWPRHLLRCVLLLGCLHLGRPRSPVTPELPGPDPTPSLTGSCPQGWASDTKLRYCYKVFSSERLQDKKSWVQAQGACQELGAQLLSLASYEEEHFVANMLNKIFGESEPEIHEQHWFWIGLNRRDPRGGQSWRWSDGVGFSYHNFDRSRHDDDDIRGCAVLDLASLQWVAMQCDTQLDWICKIPRVEPKSCDKTHTCPPCPAPELLGGPSVFLFPPKPKDTLMISRTPEVTCVVVDVSHEDPEVKFNWYVDGVEVHNAKTKPREEQYNSTYRVVSVLTVLHQDWLNGKEYKCKVSNKALPAPIEKTISKAKGQPREPQVYTLPPSRDELTKNQVSLTCLVKGFYPSDIAVEWESNGQPENNYKTTPPVLDSDGSFFLYSKLTVDKSRWQQGNVFSCSVMHEALHNHYTQKSLSLSPGK

SEQ ID NO: 46 - protein, 397 aa, Artificial Sequence
  Mature D6-Fc
RSPVTPELPGPDPTPSLTGSCPQGWASDTKLRYCYKVFSSERLQDKKSWVQAQGACQELGAQLLSLASYEEEHFVANMLNKIFGESEPEIHEQHWFWIGLNRRDPRGGQSWRWSDGVGFSYHNFDRSRHDDDDIRGCAVLDLASLQWVAMQCDTQLDWICKIPRVEPKSCDKTHTCPPCPAPELLGGPSVFLFPPKPKDTLMISRTPEVTCVVVDVSHEDPEVKFNWYVDGVEVHNAKTKPREEQYNSTYRVVSVLTVLHQDWLNGKEYKCKVSNKALPAPIEKTISKAKGQPREPQVYTLPPSRDELTKNQVSLTCLVKGFYPSDIAVEWESNGQPENNYKTTPPVLDSDGSFFLYSKLTVDKSRWQQGNVFSCSVMHEALHNHYTQKSLSLSPGK